European Patent Application EP 4 596 720 A2, published August 6, 2025. Title: ACTERIAL LEADER SEQUENCES FOR PERIPLASMIC PROTEIN EXPRESSION. Applicant: PELICAN TECHNOLOGY HOLDINGS, INC. Application EP. The sequence listing filed with the application follows.

SEQUENCE LISTING (20 sequences)

SEQ ID NO: 1 - protein, 25 aa, Pseudomonas fluorescens
MKSALKNVIPGALALLLLFPVAAQA

SEQ ID NO: 2 - protein, 18 aa, Pseudomonas fluorescens
MRQLFFCLMLMVSLTAHA

SEQ ID NO: 3 - protein, 29 aa, Pseudomonas fluorescens
MQSLPFSALRLLGVLAVMVCVLLTTPARA

SEQ ID NO: 4 - DNA, 75 bp, Pseudomonas fluorescens
  source 1..75: mol_type = other DNA
atgaaatctgcattgaagaacgttattccgggcgccctggcccttctgctgctattccccgtcgccgcccaggcc

SEQ ID NO: 5 - DNA, 54 bp, Pseudomonas fluorescens
  source 1..54: mol_type = other DNA
atgcgacaactatttttctgtttgatgctgatggtgtcgctcacggcgcacgcc

SEQ ID NO: 6 - DNA, 87 bp, Pseudomonas fluorescens
  source 1..87: mol_type = other DNA
atgcaaagcctgccgttctctgcgttacgcctgctcggtgtgctggcagtcatggtctgcgtgctgttgacgacgccagcccgtgcc

SEQ ID NO: 7 - protein, 327 aa, Erwinia chrysanthemi
ADKLPNIVILATGGTIAGSAATGTQTTGYKAGALGVDTLINAVPEVKKLANVKGEQFSNMASENMTGDVVLKLSQRVNELLARDDVDGVVITHGTDTVEESAYFLHLTVKSDKPVVFVAAMRPATAISADGPMNLLEAVRVAGDKQSRGRGVMVVLNDRIGSARYITKTNASTLDTFKANEEGYLGVIIGNRIYYQNRIDKLHTTRSVFDVRGLTSLPKVDILYGYQDDPEYLYDAAIQHGVKGIVYAGMGAGSVSVRGIAGMRKAMEKGVVVIRSTRTGNGIVPPDEELPGLVSDSLNPAHARILLMLALTRTSDPKVIQEYFHTY

SEQ ID NO: 8 - DNA, 981 bp, synthetic construct
  source 1..981: mol_type = other DNA; note = Description of Artificial Sequence: Synthetic polynucleotide
gcagacaaactccctaacatcgtaatcctcgcaactggtggtaccatcgcaggcagcgccgccaccggcacgcagaccactggctacaaggccggcgcgctgggcgtagacacgctgatcaacgccgtcccggaagtgaagaaactggccaacgtcaagggtgagcaattctccaacatggccagcgagaacatgactggcgatgtggtactgaagctctcgcagcgcgtgaacgaactgctcgcccgcgacgacgtggacggcgtggtgatcacccacggcactgataccgtcgaagagtcggcgtactttctccacctgaccgtgaagtccgataagcccgtggtgtttgtcgccgcgatgcgcccggcgaccgccatcagcgccgacgggccgatgaatctgttggaagccgtgcgcgtggcgggtgacaagcaaagccgcggtcggggcgtaatggtcgtcctgaacgatcggatcggtagcgcgcggtacatcaccaagacgaacgcctccacgctggacaccttcaaggcgaacgaagaggggtacctgggggtgatcattggcaatcgtatctattaccagaaccgcatcgacaagctgcacaccacccgctcggtgttcgacgtgcgcggtctgactagcctgcccaaggtcgacatcctgtacggctaccaagacgacccggagtacctctacgacgcggcgatccagcatggcgtgaagggcatcgtctacgccggtatgggtgccggctcggtgtcggtccgcggcatcgcgggtatgcgcaaggccatggagaaaggcgtggtcgtgattcgctcgacccggactggcaatggcatcgtaccgcccgatgaagaactcccggggctcgtgagcgatagcctcaaccccgcgcacgcccggatcctgctgatgctggcgctcacgcggaccagcgaccccaaggtcattcaagagtacttccacacctac

SEQ ID NO: 9 - protein, 326 aa, Escherichia coli
LPNITILATGGTIAGGGDSATKSNYTAGKVGVENLVNAVPQLKDIANVKGEQVVNIGSQDMNDDVWLTLAKKINTDCDKTDGFVITHGTDTMEETAYFLDLTVKCDKPVVMVGAMRPSTSMSADGPFNLYNAVVTAADKASANRGVLVVMNDTVLDGRDVTKTNTTDVATFKSVNYGPLGYIHNGKIDYQRTPARKHTSDTPFDVSKLNELPKVGIVYNYANASDLPAKALVDAGYDGIVSAGVGNGNLYKTVFDTLATAAKNGTAVVRSSRVPTGATTQDAEVDDAKYGFVASGTLNPQKARVLLQLALTQTKDPQQIQQIFNQY

SEQ ID NO: 10 - DNA, 978 bp, synthetic construct
  source 1..978: mol_type = other DNA; note = Description of Artificial Sequence: Synthetic polynucleotide
ctccctaacattactattctggccactggcggtacgattgcaggcggcggtgactcagccaccaagtcgaattacaccgccggtaaggtcggtgtcgaaaacctcgtcaacgccgtgccgcagctgaaagatatcgccaacgtcaagggcgagcaagtggtgaacatcggctcccaagatatgaacgatgacgtgtggctgacgctggccaagaaaatcaacaccgattgcgacaagacggacgggtttgtcatcacccacggcaccgacactatggaagagactgcctacttcctcgacctcacggtgaagtgcgataaaccggtagtgatggtgggcgccatgcgcccgagcacctcgatgagcgcggacggcccgttcaatctgtacaacgccgtggtaaccgcagcggacaaggcgtccgcgaaccgcggtgtattggtagtgatgaacgatacggtgctcgatgggcgcgatgtgaccaagaccaataccactgatgtggccaccttcaagagcgtgaactatggcccgctgggctacatccataacggcaagatcgattaccagcgtactcccgcccggaagcacacctcggacacccccttcgacgtgtcgaaactgaacgaactgcccaaggtcggcatcgtctacaactacgccaatgcgagcgatctgcccgcgaaggccctggtggacgccggctacgacgggatcgtatcggcgggtgtgggcaatggtaacctgtacaagaccgtgtttgacaccctggcgacggcggcgaagaacggcaccgccgtggtccgcagcagccgcgtgcccactggggcgaccacccaagacgccgaggtcgacgacgcgaagtacggcttcgtagccagcggcaccctgaacccgcaaaaggcccgggtcctgctgcagctggcgctcacgcagacgaaggacccgcagcaaatccaacagatcttcaaccagtac

SEQ ID NO: 11-19 - skipped (9 entries)

SEQ ID NO: 20 - DNA, 1020 bp, synthetic construct
  source 1..1020: mol_type = other DNA; note = Description of Artificial Sequence: Synthetic polynucleotide
atatgctcttcagccgcagacaaactccctaacatcgtaatcctcgcaactggtggtaccatcgcaggcagcgccgccaccggcacgcagaccactggctacaaggccggcgcgctgggcgtagacacgctgatcaacgccgtcccggaagtgaagaaactggccaacgtcaagggtgagcaattctccaacatggccagcgagaacatgactggcgatgtggtactgaagctctcgcagcgcgtgaacgaactgctcgcccgcgacgacgtggacggcgtggtgatcacccacggcactgataccgtcgaagagtcggcgtactttctccacctgaccgtgaagtccgataagcccgtggtgtttgtcgccgcgatgcgcccggcgaccgccatcagcgccgacgggccgatgaatctgttggaagccgtgcgcgtggcgggtgacaagcaaagccgcggtcggggcgtaatggtcgtcctgaacgatcggatcggtagcgcgcggtacatcaccaagacgaacgcctccacgctggacaccttcaaggcgaacgaagaggggtacctgggggtgatcattggcaatcgtatctattaccagaaccgcatcgacaagctgcacaccacccgctcggtgttcgacgtgcgcggtctgactagcctgcccaaggtcgacatcctgtacggctaccaagacgacccggagtacctctacgacgcggcgatccagcatggcgtgaagggcatcgtctacgccggtatgggtgccggctcggtgtcggtccgcggcatcgcgggtatgcgcaaggccatggagaaaggcgtggtcgtgattcgctcgacccggactggcaatggcatcgtaccgcccgatgaagaactcccggggctcgtgagcgatagcctcaaccccgcgcacgcccggatcctgctgatgctggcgctcacgcggaccagcgaccccaaggtcattcaagagtacttccacacctactgataatagttcagaagagcatat